European Patent Specification EP 3 374 506 B1, published December 27, 2023. Title: ogenous Control of Mammalian Gene Expression Through Aptamer-Mediated Modulation of Polyadenylation. Applicant: Yen, Laising Luo, Liming Chao, Pei-Wen. Application UNKNOWN. The sequence listing filed with the application follows.

SEQUENCE LISTING (61 sequences)

SEQ ID NO: 1 - RNA, 50 nt, Artificial Sequence
  Synthetic Primer
ucccacuguccuuuccuaauaaaaugaggaaauugcaucgcauugucuga

SEQ ID NO: 2 - RNA, 93 nt, Artificial Sequence
  Synthetic Primer
ucagacaaugcgaugcaauuucgagcucucgcgaggugccacuccccacuguccuuuccuaauaaaaugaggaaauugcaucgcauugucuga

SEQ ID NO: 3 - RNA, 12 nt, Artificial Sequence
  Synthetic Primer
aauaaaaauaaa

SEQ ID NO: 4 - RNA, 71 nt, Artificial Sequence
  Synthetic Primer
gggccuaaaacauaccagaucgccacccgcgcuuuaaucuggagaggugaagaauacgaccaccuaggcuc

SEQ ID NO: 5 - RNA, 12 nt, Artificial Sequence
  Synthetic Primer
aauaaaaauaaa

SEQ ID NO: 6 - RNA, 12 nt, Artificial Sequence
  Synthetic Primer
cacacaaauaaa

SEQ ID NO: 7 - RNA, 12 nt, Artificial Sequence
  Synthetic Primer
aaauaaacacac

SEQ ID NO: 8 - RNA, 92 nt, Artificial Sequence
  Synthetic Primer
cacagaucuggagaggugaagaauacgaccaccugcguuuuauacuuuguaacacaaauaaaguauaaagugcaaaacauaccagaucugug

SEQ ID NO: 9 - RNA, 92 nt, Artificial Sequence
  Synthetic Primer
cacagaucuggagaggugaagaauacgaccaccugcguuauauacuuuguaacacaaauaaaguauauagugcaaaacauaccagaucugug

SEQ ID NO: 10 - DNA, 27 bp, Artificial Sequence
  Synthetic Primer
gtgcaaaacaaaaaaaaaaaaaaaaaa

SEQ ID NO: 11 - DNA, 27 bp, Artificial Sequence
  Synthetic Primer
gtgcaaaacataaaaaaaaaaaaaaaa

SEQ ID NO: 12 - DNA, 28 bp, Artificial Sequence
  Synthetic Primer
gtgcaaaacataccaaaaaaaaaaaaaa

SEQ ID NO: 13 - RNA, 92 nt, Artificial Sequence; identical to SEQ ID NO: 8
  Synthetic Primer

SEQ ID NO: 14 - RNA, 11 nt, Artificial Sequence
  Synthetic Primer
aaaacauacca

SEQ ID NO: 15 - RNA, 92 nt, Artificial Sequence; identical to SEQ ID NO: 8
  Synthetic Primer

SEQ ID NO: 16 - RNA, 92 nt, Artificial Sequence
  Synthetic Primer
cacagaucuggggaggugaagaauacgaccaccugcguuuuauacuuuguaacacaaauaaaguauaaagugcaaaacauaccagaucugug

SEQ ID NO: 17 - RNA, 92 nt, Artificial Sequence
  Synthetic Primer
cacaaaucuggggaggugaagaauacgaccaccugcguuuuauacuuuguaacacaaauaaaguauaaagugcaaaacauaccagaucugug

SEQ ID NO: 18 - DNA, 92 bp, Artificial Sequence
  Synthetic Primer
cacaaaucuggggaggugaagaauacgaccaccugcuaguuauacuuuguaacacaaauaaaguauagctagcaaaacauaccagaucugug

SEQ ID NO: 19 - RNA, 92 nt, Artificial Sequence; identical to SEQ ID NO: 17
  Synthetic Primer

SEQ ID NO: 20 - DNA, 92 bp, Artificial Sequence; identical to SEQ ID NO: 18
  Synthetic Primer

SEQ ID NO: 21 - DNA, 92 bp, Artificial Sequence; identical to SEQ ID NO: 18
  Synthetic Primer

SEQ ID NO: 22 - RNA, 12 nt, Artificial Sequence
  Synthetic Primer
ccaacccccgca

SEQ ID NO: 23 - RNA, 11 nt, Artificial Sequence
  Synthetic Primer
uuugcuuagaa

SEQ ID NO: 24 - RNA, 12 nt, Artificial Sequence
  Synthetic Primer
ccgucuccccca

SEQ ID NO: 25 - RNA, 12 nt, Artificial Sequence
  Synthetic Primer
ggggccucgaga

SEQ ID NO: 26 - RNA, 97 nt, Artificial Sequence
  Synthetic Primer
cacagaucuggggaggugaagaauacgaccaccugcguuuuauacuuuguuggaacacaccaauaaaguauaaagugcaaaacauaccagaucugug

SEQ ID NO: 27 - DNA, 92 bp, Artificial Sequence
  Synthetic Primer
cacaaaucuggggaggugaagaauacgaccaccugcuaguuacgcuuuguaacacaaauaaagcguagctagcaaaacauaccagaucugug

SEQ ID NO: 28 - RNA, 136 nt, Artificial Sequence
  Synthetic Primer
cacaaaucuggggaggugaagaauacgaccaccugcguuuuauacuuuguuaaaacauaccagaucgaaagaucuggggaggugaagaauacgaccaccuaauaaaguauaaagugcaaaacauaccagaucugug

SEQ ID NO: 29 - RNA, 10 nt, Artificial Sequence
  Synthetic Primer
aucgaaagau

SEQ ID NO: 30 - RNA, 10 nt, Artificial Sequence
  Synthetic Primer
auugaaagau

SEQ ID NO: 31 - DNA, 21 bp, Artificial Sequence
  Synthetic Peptide
accagatcgaaagatctgggg

SEQ ID NO: 32 - DNA, 21 bp, Artificial Sequence
  Synthetic Peptide
accagatcgatcgatctgggg

SEQ ID NO: 33 - DNA, 19 bp, Artificial Sequence
  Synthetic Peptide
accagatcgcgatctgggg

SEQ ID NO: 34 - DNA, 17 bp, Artificial Sequence
  Synthetic Primer
accagatcgatctgggg

SEQ ID NO: 35 - DNA, 22 bp, Artificial Sequence
  Synthetic Primer
accagatcgattcgatctgggg

SEQ ID NO: 36 - DNA, 15 bp, Artificial Sequence
  Synthetic Primer
accagatatctgggg

SEQ ID NO: 37 - DNA, 23 bp, Artificial Sequence
  Synthetic Primer
accagatcgaattcgatctgggg

SEQ ID NO: 38 - DNA, 24 bp, Artificial Sequence
  Synthetic Primer
accagatcgaatttcgatctgggg

SEQ ID NO: 39 - DNA, 25 bp, Artificial Sequence
  Synthetic Primer
accagatcgaatattcgatctgggg

SEQ ID NO: 40 - DNA, 26 bp, Artificial Sequence
  Synthetic Primer
accagatcgaatcattcgatctgggg

SEQ ID NO: 41 - DNA, 27 bp, Artificial Sequence
  Synthetic Primer
accagatcgaatcgattcgatctgggg

SEQ ID NO: 42 - DNA, 27 bp, Artificial Sequence
  Synthetic Primer
accagattacccttgggtgatctgggg

SEQ ID NO: 43 - DNA, 28 bp, Artificial Sequence
  Synthetic Primer
accagatcgaatctgattcgatctgggg

SEQ ID NO: 44 - DNA, 41 bp, Artificial Sequence
  Synthetic Primer
accatcctaagcctaaggcaaacgctatggtatggatgggg

SEQ ID NO: 45 - DNA, 21 bp, Artificial Sequence
  Synthetic Primer
accagatcgaaagatctgggg

SEQ ID NO: 46 - DNA, 21 bp, Artificial Sequence
  Synthetic Primer
accagatcgatcgatctgggg

SEQ ID NO: 47 - DNA, 19 bp, Artificial Sequence
  Synthetic Primer
accagatcgcgatctgggg

SEQ ID NO: 48 - DNA, 17 bp, Artificial Sequence
  Synthetic Primer
accagatcgatctgggg

SEQ ID NO: 49 - DNA, 22 bp, Artificial Sequence
  Synthetic Primer
accagatcgaatcgatctgggg

SEQ ID NO: 50 - DNA, 15 bp, Artificial Sequence
  Synthetic Primer
accagatatctgggg

SEQ ID NO: 51 - DNA, 23 bp, Artificial Sequence
  Synthetic Primer
accagatcgaattcgatctgggg

SEQ ID NO: 52 - DNA, 24 bp, Artificial Sequence
  Synthetic Primer
accagatcgaaattcgatctgggg

SEQ ID NO: 53 - DNA, 25 bp, Artificial Sequence
  Synthetic Primer
accagatcgaatattcgatctgggg

SEQ ID NO: 54 - DNA, 26 bp, Artificial Sequence
  Synthetic Primer
accagatcgaatgattcgatctgggg

SEQ ID NO: 55 - DNA, 27 bp, Artificial Sequence
  Synthetic Primer
accagatcgaatcgattcgatctgggg

SEQ ID NO: 56 - DNA, 27 bp, Artificial Sequence
  Synthetic Primer
accagattacccgagggtgatctgggg

SEQ ID NO: 57 - DNA, 28 bp, Artificial Sequence
  Synthetic Primer
accagatcgaatcagattcgatctgggg

SEQ ID NO: 58 - DNA, 21 bp, Artificial Sequence
  Synthetic Primer
accagatcgaaagatctgggg

SEQ ID NO: 59 - DNA, 370 bp, Artificial Sequence
  Synthetic Primerr
gctagccacacacacaaatctggggaggtgaagaatacgaccacctgcgttttatactttgttaaaacataccagatcgaaagatctggggaggtgaagaatacgaccacctaataaagtataaagtgcaaaacataccagatctgtgtgttggttttttgtgtggaattccacacacacaaatctggggaggtgaagaatacgaccacctgcgttttatactttgttaaaacataccagatcgaaagatctggggaggtgaagaatacgaccacctaataaagtataaagtgcaaaacataccagatctgtgtgttggttttttgtgtgaacgggggagggggaggaaagggggagggggagcggccgc

SEQ ID NO: 60 - DNA, 374 bp, Artificial Sequence
  Synthetic Primer
ctgcagcacacacacaaatctggggaggtgaagaatacgaccacctgcgttttatactttgttaaaacataccagatcgaattcgatctggggaggtgaagaatacgaccacctaataaagtataaagtgcaaaacataccagatctgtgtgttggttttttgtgtggctagccacacacacaaatctggggaggtgaagaatacgaccacctgcgttttatactttgttaaaacataccagatcgaattcgatctggggaggtgaagaatacgaccacctaataaagtataaagtgcaaaacataccagatctgtgtgttggttttttgtgtgaacgggggagggggaggaaagggggagggggagcggccgc

SEQ ID NO: 61 - DNA, 396 bp, Artificial Sequence
  Synthetic Primer
gctagcgaattgcacacacacaaatctggggaggtgaagaatacgaccacctgcgttttatactttgttaaaacataccatcctaagcctaaggcaaacgctatggtatggatggggaggtgaagaatacgaccacctaataaagtataaagtgcaaaacataccagatctgtgtgttggttttttgtgtggaattccacacacacaaatctggggaggtgaagaatacgaccacctgcgttttatactttgttaaaacataccagatcgaaagatctggggaggtgaagaatacgaccacctaataaagtataaagtgcaaaacataccagatctgtgtgttggttttttgtgtgaacgggggagggggaggaaagggggagggggagcggccgc